European Patent Specification EP 3 277 099 B1, published November 8, 2023. Title: HIGH EFFICIENCY OXALATE-DEGRADING ENZYMES FOR DEGRADATION OF INSOLUBLE AND SOLUBLE OXALATE. Applicant: CAPTOZYME, LLC. Application PCT/US2016/025937. The sequence listing filed with the application follows.

SEQUENCE LISTING (53 sequences)

SEQ ID NO: 1 - protein, 398 aa, Bacillus cereus
MKKRTVNEAGRNVPQPIRSDGAGAIDSGPRNVMRDIQNPNMLVPPITDAGLVPNLKFSFSDTSMILKQGGWSREITARELPVSTTIAGVNMSLTAGGVRELHWHKEAEWAYMLLGRARITAVDQNGRNFIADVGPGDLWYFPPGIPHSIQGLEHCEFLLVFDDGHFSDLSTLAISDWFAHTPKEVLSANFGVPESVFRSLPSDQVYIYQGEVPGSLESQEVQSPKGEVPLTFKHELLKQKPVKTPGGSVRIVDSTNFPISKTIAAALVEVEPGGMRELHWHPNNDEWQYYLTGEARMTVFLGNGTARTFDYRAGDVGYVPFATGHYIQNTGTETLWFLEMFRSNRFEDVSLNQWMALTPKEIVESNIHVGPQVMDSLRKEKWPVVKYPGFSYSPKSDE

SEQ ID NO: 2 - protein, 389 aa, Synechococcus elongatus
MQKKSKFFLGLLGVITCFVLIGSFCLPSLAQTQTWRSLSNVVWGKDLPAFSYPFSKTPLVDYDGGVTKQVGTYNFPVSKGMAGVYMTLKPGAIRELHWHANAAEWAYVIEGRTRVTLTNPDGQVQIADVDQGGLWYFPRGWGHSIEGIGPGTAKFLLVFNDGTFSEGATFSITDWLSHTPISWVQQNFGWSQDEVEKLPKKQVYISRYNPEVKPLDKTQSRNPKVSRIVLPYTHNLLAEKPRTSQAGNTLKLASAKEFPASFNMAGALLRLEPGAMRQLHWHPNADEWQYVLNGSMDLAVFASEGKASMSRLQKGDVGYVPKGYGHALRNSSDQPLDVLIVFNDGDYQSIDLNDWIMSNPNTVLDDVFQLSPQLLDKLPKESEILIPRS

SEQ ID NO: 3 - protein, 360 aa, Synechococcus elongatus
MQTQTWRSLSNVVWGKDLPAFSYPFSKTPLVDYDGGVTKQVGTYNFPVSKGMAGVYMTLKPGAIRELHWHANAAEWAYVIEGRTRVTLTNPDGQVQIADVDQGGLWYFPRGWGHSIEGIGPGTAKFLLVFNDGTFSEGATFSITDWLSHTPISWVQQNFGWSQDEVEKLPKKQVYISRYNPEVKPLDKTQSRNPKVSRIVLPYTHNLLAEKPRTSQAGNTLKLASAKEFPASFNMAGALLRLEPGAMRQLHWHPNADEWQYVLNGSMDLAVFASEGKASMSRLQKGDVGYVPKGYGHALRNSSDQPLDVLIVFNDGDYQSIDLNDWIMSNPNTVLDDVFQLSPQLLDKLPKESEILIPRS

SEQ ID NO: 4 - protein, 379 aa, Synechococcus elongatus
MLGVITCFVLIGSFCLPSLAQTQTWRSLSNVVWGKDLPAFSYPFSKTPLVDYDGGVTKQVGTYNFPVSKGMAGVYMTLKPGAIRELHWHANAAEWAYVIEGRTRVTLTNPDGQVQIADVDQGGLWYFPRGWGHSIEGIGPGTAKFLLVFNDGTFSEGATFSITDWLSHTPISWVQQNFGWSQDEVEKLPKKQVYISRYNPEVKPLDKTQSRNPKVSRIVLPYTHNLLAEKPRTSQAGNTLKLASAKEFPASFNMAGALLRLEPGAMRQLHWHPNADEWQYVLNGSMDLAVFASEGKASMSRLQKGDVGYVPKGYGHALRNSSDQPLDVLIVFNDGDYQSIDLNDWIMSNPNTVLDDVFQLSPQLLDKLPKESEILIPRS

SEQ ID NO: 5 - protein, 393 aa, Bacillus cereus
MKKRTVNEAGRNVPQPIRSDGAGAIDSGPRNVMRQTQTWRSLSNVVWGKDLPAFSYPFSKTPLVDYDGGVTKQVGTYNFPVSKGMAGVYMTLKPGAIRELHWHANAAEWAYVIEGRTRVTLTNPDGQVQIADVDQGGLWYFPRGWGHSIEGIGPGTAKFLLVFNDGTFSEGATFSITDWLSHTPISWVQQNFGWSQDEVEKLPKKQVYISRYNPEVKPLDKTQSRNPKVSRIVLPYTHNLLAEKPRTSQAGNTLKLASAKEFPASFNMAGALLRLEPGAMRQLHWHPNADEWQYVLNGSMDLAVFASEGKASMSRLQKGDVGYVPKGYGHALRNSSDQPLDVLIVFNDGDYQSIDLNDWIMSNPNTVLDDVFQLSPQLLDKLPKESEILIPRS

SEQ ID NO: 6 - protein, 369 aa, Synechococcus elongatus
MGSFCLPSLAQTQTWRSLSNVVWGKDLPAFSYPFSKTPLVDYDGGVTKQVGTYNFPVSKGMAGVYMTLKPGAIRELHWHANAAEWAYVIEGRTRVTLTNPDGQVQIADVDQGGLWYFPRGWGHSIEGIGPGTAKFLLVFNDGTFSEGATFSITDWLSHTPISWVQQNFGWSQDEVEKLPKKQVYISRYNPEVKPLDKTQSRNPKVSRIVLPYTHNLLAEKPRTSQAGNTLKLASAKEFPASFNMAGALLRLEPGAMRQLHWHPNADEWQYVLNGSMDLAVFASEGKASMSRLQKGDVGYVPKGYGHALRNSSDQPLDVLIVFNDGDYQSIDLNDWIMSNPNTVLDDVFQLSPQLLDKLPKESEILIPRS

SEQ ID NO: 7 - protein, 369 aa, Synechococcus elongatus
MGSFNLPSLAQTQTWRSLSNVVWGKDLPAFSYPFSKTPLVDYDGGVTKQVGTYNFPVSKGMAGVYMTLKPGAIRELHWHANAAEWAYVIEGRTRVTLTNPDGQVQIADVDQGGLWYFPRGWGHSIEGIGPGTAKFLLVFNDGTFSEGATFSITDWLSHTPISWVQQNFGWSQDEVEKLPKKQVYISRYNPEVKPLDKTQSRNPKVSRIVLPYTHNLLAEKPRTSQAGNTLKLASAKEFPASFNMAGALLRLEPGAMRQLHWHPNADEWQYVLNGSMDLAVFASEGKASMSRLQKGDVGYVPKGYGHALRNSSDQPLDVLIVFNDGDYQSIDLNDWIMSNPNTVLDDVFQLSPQLLDKLPKESEILIPRS

SEQ ID NO: 8 - protein, 369 aa, Synechococcus elongatus
MGSFSLPSLAQTQTWRSLSNVVWGKDLPAFSYPFSKTPLVDYDGGVTKQVGTYNFPVSKGMAGVYMTLKPGAIRELHWHANAAEWAYVIEGRTRVTLTNPDGQVQIADVDQGGLWYFPRGWGHSIEGIGPGTAKFLLVFNDGTFSEGATFSITDWLSHTPISWVQQNFGWSQDEVEKLPKKQVYISRYNPEVKPLDKTQSRNPKVSRIVLPYTHNLLAEKPRTSQAGNTLKLASAKEFPASFNMAGALLRLEPGAMRQLHWHPNADEWQYVLNGSMDLAVFASEGKASMSRLQKGDVGYVPKGYGHALRNSSDQPLDVLIVFNDGDYQSIDLNDWIMSNPNTVLDDVFQLSPQLLDKLPKESEILIPRS

SEQ ID NO: 9 - protein, 369 aa, Synechococcus elongatus
MGSFALPSLAQTQTWRSLSNVVWGKDLPAFSYPFSKTPLVDYDGGVTKQVGTYNFPVSKGMAGVYMTLKPGAIRELHWHANAAEWAYVIEGRTRVTLTNPDGQVQIADVDQGGLWYFPRGWGHSIEGIGPGTAKFLLVFNDGTFSEGATFSITDWLSHTPISWVQQNFGWSQDEVEKLPKKQVYISRYNPEVKPLDKTQSRNPKVSRIVLPYTHNLLAEKPRTSQAGNTLKLASAKEFPASFNMAGALLRLEPGAMRQLHWHPNADEWQYVLNGSMDLAVFASEGKASMSRLQKGDVGYVPKGYGHALRNSSDQPLDVLIVFNDGDYQSIDLNDWIMSNPNTVLDDVFQLSPQLLDKLPKESEILIPRS

SEQ ID NO: 10 - protein, 389 aa, Synechococcus elongatus
MQKKSKFFLGLLGVITCFVLIGSFCLPSLAQTQTWRSLSNVVWGKDLPAFSYPFSKTPLVDYDGGVTKQVGTYNFPVSKGMAGVYMTLKPGAIRELHWHANAAEWAYVIEGRTRVTLTNPDGQVQIADVDQGGLWYFPRGWGHSIEGIGPGTAKFLLVFNDGTFSENSTFQLTDWLSHTPISWVQQNFGWSQDEVEKLPKKQVYISRYNPEVKPLDKTQSRNPKVSRIVLPYTHNLLAEKPRTSQAGNTLKLASAKEFPASFNMAGALLRLEPGAMRQLHWHPNADEWQYVLNGSMDLAVFASEGKASMSRLQKGDVGYVPKGYGHALRNSSDQPLDVLIVFNDGDYQSIDLNDWIMSNPNTVLDDVFQLSPQLLDKLPKESEILIPRS

SEQ ID NO: 11 - protein, 389 aa, Synechococcus elongatus
MQKKSKFFLGLLGVITCFVLIGSFCLPSLAQTQTWRSLSNVVWGKDLPAFSYPFSKTPLVDYDGGVTKQVGTYNFPVSKGMAGVYMTLKPGAIRELHWHANAAEWAYVIEGRTRVTLTNPDGQVQIADVDQGGLWYFPRGWGHSIEGIGPGTAKFLLVFNDGTFSEGATFSITDWLSHTPISWVQQNFGWSQDEVEKLPKKQVYISRYNPEVKPLDKTQSRNPKVSRIVLPYTHNLLAEKPRTSQAGNTLKLASAKEFPASFNMAGALLRLEPGAMRQLHWHPNADEWQYVLNGSMDLAVFASEGKASMSRLQKGDVGYVPKGYGHALRNSSDQPLDVLEVFNDGDYQSIDLNDWIMSNPNTVLDDVFQLSPQLLDKLPKESEILIPRS

SEQ ID NO: 12 - protein, 389 aa, Synechococcus elongatus
MQKKSKFFLGLLGVITCFVLIGSFCLPSLAQTQTWRSLSNVVWGKDLPAFSYPFSKTPLVDYDGGVTKQVGTYNFPVSKGMAGVYMTLKPGAIRELHWHANAAEWAYVIEGRTRVTLTNPDGQVQIADVDQGGLWYFPRGWGHSIEGIGPGTAKFLLVFNDGTFSENSTFQLTDWLSHTPISWVQQNFGWSQDEVEKLPKKQVYISRYNPEVKPLDKTQSRNPKVSRIVLPYTHNLLAEKPRTSQAGNTLKLASAKEFPASFNMAGALLRLEPGAMRQLHWHPNADEWQYVLNGSMDLAVFASEGKASMSRLQKGDVGYVPKGYGHALRNSSDQPLDVLEVFNDGDYQSIDLNDWIMSNPNTVLDDVFQLSPQLLDKLPKESEILIPRS

SEQ ID NO: 13 - protein, 389 aa, Synechococcus elongatus
MQKKSKFFLGLLGVITCFVLIGSFCLPSLAQTQTWRSLSNVVWGKDLPAFSYPFSKTPLVDYDGGVTKQVGTYNFPVSKGMAGVYMTLKPGAIRELHWHANAAEWAYVIEGRTRVTLTNPDGQVQIADVDQGGLWYFPRGWGHSIEGIGPGTAKFLLVFNDGTFSEGATFSITDWLSHTPISWVQQNFGWSQDEVEKLPKKQVYISRYNPEVKPLDKTQSRNPKVSRIVLPYTHNLLAEKPRTSQAGNTLKLASAKEFPASFNMAGALLRLEPGAMRQLHWHPNADEWQYVLNGSMDLAVFASEGKASMSRLQKGDVGYVPKGYGHALRNSSDQPLDVLAVFNDGDYQSIDLNDWIMSNPNTVLDDVFQLSPQLLDKLPKESEILIPRS

SEQ ID NO: 14 - protein, 389 aa, Synechococcus elongatus
MQKKSKFFLGLLGVITCFVLIGSFCLPSLAQTQTWRSLSNVVWGKDLPAFSYPFSKTPLVDYDGGVTKQVGTYNFPVSKGMAGVYMTLKPGAIRELHWHANAAEWAYVIEGRTRVTLTNPDGQVQIADVDQGGLWYFPRGWGHSIEGIGPGTAKFLLVFNDGTFSEGATFSITDWLSHTPISWVQQNFGWSQDEVEKLPKKQVYISRYNPEVKPLDKTQSRNPKVSRIVLPYTHNLLAEKPRTSQAGNTLKLASAKEFPASFNMAGALLRLEPGAMRQLHWHPNADEWQYVLNGSMDLAVFASEGKASMSRLQKGDVGYVPKGYGHALRNSSDQPLDVLCVFNDGDYQSIDLNDWIMSNPNTVLDDVFQLSPQLLDKLPKESEILIPRS

SEQ ID NO: 15 - protein, 389 aa, Synechococcus elongatus
MQKKSKFFLGLLGVITCFVLIGSFCLPSLAQTQTWRSLSNVVWGKDLPAFSYPFSKTPLVDYDGGVTKQVGTYNFPVSKGMAGVYMTLKPGAIRELHWHANAAEWAYVIEGRTRVTLTNPDGQVQIADVDQGGLWYFPRGWGHSIEGIGPGTAKFLLVFNDGTFSEGATFSITDWLSHTPISWVQQNFGWSQDEVEKLPKKQVYISRYNPEVKPLDKTQSRNPKVSRIVLPYTHNLLAEKPRTSQAGNTLKLASAKEFPASFNMAGALLRLEPGAMRQLHWHPNADEWQYVLNGSMDLAVFASEGKASMSRLQKGDVGYVPKGYGHALRNSSDQPLDVLDVFNDGDYQSIDLNDWIMSNPNTVLDDVFQLSPQLLDKLPKESEILIPRS

SEQ ID NO: 16 - protein, 389 aa, Synechococcus elongatus; identical to SEQ ID NO: 11

SEQ ID NO: 17 - protein, 389 aa, Synechococcus elongatus
MQKKSKFFLGLLGVITCFVLIGSFCLPSLAQTQTWRSLSNVVWGKDLPAFSYPFSKTPLVDYDGGVTKQVGTYNFPVSKGMAGVYMTLKPGAIRELHWHANAAEWAYVIEGRTRVTLTNPDGQVQIADVDQGGLWYFPRGWGHSIEGIGPGTAKFLLVFNDGTFSEGATFSITDWLSHTPISWVQQNFGWSQDEVEKLPKKQVYISRYNPEVKPLDKTQSRNPKVSRIVLPYTHNLLAEKPRTSQAGNTLKLASAKEFPASFNMAGALLRLEPGAMRQLHWHPNADEWQYVLNGSMDLAVFASEGKASMSRLQKGDVGYVPKGYGHALRNSSDQPLDVLFVFNDGDYQSIDLNDWIMSNPNTVLDDVFQLSPQLLDKLPKESEILIPRS

SEQ ID NO: 18 - protein, 389 aa, Synechococcus elongatus
MQKKSKFFLGLLGVITCFVLIGSFCLPSLAQTQTWRSLSNVVWGKDLPAFSYPFSKTPLVDYDGGVTKQVGTYNFPVSKGMAGVYMTLKPGAIRELHWHANAAEWAYVIEGRTRVTLTNPDGQVQIADVDQGGLWYFPRGWGHSIEGIGPGTAKFLLVFNDGTFSEGATFSITDWLSHTPISWVQQNFGWSQDEVEKLPKKQVYISRYNPEVKPLDKTQSRNPKVSRIVLPYTHNLLAEKPRTSQAGNTLKLASAKEFPASFNMAGALLRLEPGAMRQLHWHPNADEWQYVLNGSMDLAVFASEGKASMSRLQKGDVGYVPKGYGHALRNSSDQPLDVLGVFNDGDYQSIDLNDWIMSNPNTVLDDVFQLSPQLLDKLPKESEILIPRS

SEQ ID NO: 19 - protein, 389 aa, Synechococcus elongatus
MQKKSKFFLGLLGVITCFVLIGSFCLPSLAQTQTWRSLSNVVWGKDLPAFSYPFSKTPLVDYDGGVTKQVGTYNFPVSKGMAGVYMTLKPGAIRELHWHANAAEWAYVIEGRTRVTLTNPDGQVQIADVDQGGLWYFPRGWGHSIEGIGPGTAKFLLVFNDGTFSEGATFSITDWLSHTPISWVQQNFGWSQDEVEKLPKKQVYISRYNPEVKPLDKTQSRNPKVSRIVLPYTHNLLAEKPRTSQAGNTLKLASAKEFPASFNMAGALLRLEPGAMRQLHWHPNADEWQYVLNGSMDLAVFASEGKASMSRLQKGDVGYVPKGYGHALRNSSDQPLDVLHVFNDGDYQSIDLNDWIMSNPNTVLDDVFQLSPQLLDKLPKESEILIPRS

SEQ ID NO: 20 - protein, 389 aa, Synechococcus elongatus
MQKKSKFFLGLLGVITCFVLIGSFCLPSLAQTQTWRSLSNVVWGKDLPAFSYPFSKTPLVDYDGGVTKQVGTYNFPVSKGMAGVYMTLKPGAIRELHWHANAAEWAYVIEGRTRVTLTNPDGQVQIADVDQGGLWYFPRGWGHSIEGIGPGTAKFLLVFNDGTFSEGATFSITDWLSHTPISWVQQNFGWSQDEVEKLPKKQVYISRYNPEVKPLDKTQSRNPKVSRIVLPYTHNLLAEKPRTSQAGNTLKLASAKEFPASFNMAGALLRLEPGAMRQLHWHPNADEWQYVLNGSMDLAVFASEGKASMSRLQKGDVGYVPKGYGHALRNSSDQPLDVLKVFNDGDYQSIDLNDWIMSNPNTVLDDVFQLSPQLLDKLPKESEILIPRS

SEQ ID NO: 21 - protein, 389 aa, Synechococcus elongatus
MQKKSKFFLGLLGVITCFVLIGSFCLPSLAQTQTWRSLSNVVWGKDLPAFSYPFSKTPLVDYDGGVTKQVGTYNFPVSKGMAGVYMTLKPGAIRELHWHANAAEWAYVIEGRTRVTLTNPDGQVQIADVDQGGLWYFPRGWGHSIEGIGPGTAKFLLVFNDGTFSEGATFSITDWLSHTPISWVQQNFGWSQDEVEKLPKKQVYISRYNPEVKPLDKTQSRNPKVSRIVLPYTHNLLAEKPRTSQAGNTLKLASAKEFPASFNMAGALLRLEPGAMRQLHWHPNADEWQYVLNGSMDLAVFASEGKASMSRLQKGDVGYVPKGYGHALRNSSDQPLDVLLVFNDGDYQSIDLNDWIMSNPNTVLDDVFQLSPQLLDKLPKESEILIPRS

SEQ ID NO: 22 - protein, 389 aa, Synechococcus elongatus
MQKKSKFFLGLLGVITCFVLIGSFCLPSLAQTQTWRSLSNVVWGKDLPAFSYPFSKTPLVDYDGGVTKQVGTYNFPVSKGMAGVYMTLKPGAIRELHWHANAAEWAYVIEGRTRVTLTNPDGQVQIADVDQGGLWYFPRGWGHSIEGIGPGTAKFLLVFNDGTFSEGATFSITDWLSHTPISWVQQNFGWSQDEVEKLPKKQVYISRYNPEVKPLDKTQSRNPKVSRIVLPYTHNLLAEKPRTSQAGNTLKLASAKEFPASFNMAGALLRLEPGAMRQLHWHPNADEWQYVLNGSMDLAVFASEGKASMSRLQKGDVGYVPKGYGHALRNSSDQPLDVLMVFNDGDYQSIDLNDWIMSNPNTVLDDVFQLSPQLLDKLPKESEILIPRS

SEQ ID NO: 23 - protein, 389 aa, Synechococcus elongatus
MQKKSKFFLGLLGVITCFVLIGSFCLPSLAQTQTWRSLSNVVWGKDLPAFSYPFSKTPLVDYDGGVTKQVGTYNFPVSKGMAGVYMTLKPGAIRELHWHANAAEWAYVIEGRTRVTLTNPDGQVQIADVDQGGLWYFPRGWGHSIEGIGPGTAKFLLVFNDGTFSEGATFSITDWLSHTPISWVQQNFGWSQDEVEKLPKKQVYISRYNPEVKPLDKTQSRNPKVSRIVLPYTHNLLAEKPRTSQAGNTLKLASAKEFPASFNMAGALLRLEPGAMRQLHWHPNADEWQYVLNGSMDLAVFASEGKASMSRLQKGDVGYVPKGYGHALRNSSDQPLDVLNVFNDGDYQSIDLNDWIMSNPNTVLDDVFQLSPQLLDKLPKESEILIPRS

SEQ ID NO: 24 - protein, 389 aa, Synechococcus elongatus
MQKKSKFFLGLLGVITCFVLIGSFCLPSLAQTQTWRSLSNVVWGKDLPAFSYPFSKTPLVDYDGGVTKQVGTYNFPVSKGMAGVYMTLKPGAIRELHWHANAAEWAYVIEGRTRVTLTNPDGQVQIADVDQGGLWYFPRGWGHSIEGIGPGTAKFLLVFNDGTFSEGATFSITDWLSHTPISWVQQNFGWSQDEVEKLPKKQVYISRYNPEVKPLDKTQSRNPKVSRIVLPYTHNLLAEKPRTSQAGNTLKLASAKEFPASFNMAGALLRLEPGAMRQLHWHPNADEWQYVLNGSMDLAVFASEGKASMSRLQKGDVGYVPKGYGHALRNSSDQPLDVLPVFNDGDYQSIDLNDWIMSNPNTVLDDVFQLSPQLLDKLPKESEILIPRS

SEQ ID NO: 25 - protein, 389 aa, Synechococcus elongatus
MQKKSKFFLGLLGVITCFVLIGSFCLPSLAQTQTWRSLSNVVWGKDLPAFSYPFSKTPLVDYDGGVTKQVGTYNFPVSKGMAGVYMTLKPGAIRELHWHANAAEWAYVIEGRTRVTLTNPDGQVQIADVDQGGLWYFPRGWGHSIEGIGPGTAKFLLVFNDGTFSEGATFSITDWLSHTPISWVQQNFGWSQDEVEKLPKKQVYISRYNPEVKPLDKTQSRNPKVSRIVLPYTHNLLAEKPRTSQAGNTLKLASAKEFPASFNMAGALLRLEPGAMRQLHWHPNADEWQYVLNGSMDLAVFASEGKASMSRLQKGDVGYVPKGYGHALRNSSDQPLDVLQVFNDGDYQSIDLNDWIMSNPNTVLDDVFQLSPQLLDKLPKESEILIPRS

SEQ ID NO: 26 - protein, 389 aa, Synechococcus elongatus
MQKKSKFFLGLLGVITCFVLIGSFCLPSLAQTQTWRSLSNVVWGKDLPAFSYPFSKTPLVDYDGGVTKQVGTYNFPVSKGMAGVYMTLKPGAIRELHWHANAAEWAYVIEGRTRVTLTNPDGQVQIADVDQGGLWYFPRGWGHSIEGIGPGTAKFLLVFNDGTFSEGATFSITDWLSHTPISWVQQNFGWSQDEVEKLPKKQVYISRYNPEVKPLDKTQSRNPKVSRIVLPYTHNLLAEKPRTSQAGNTLKLASAKEFPASFNMAGALLRLEPGAMRQLHWHPNADEWQYVLNGSMDLAVFASEGKASMSRLQKGDVGYVPKGYGHALRNSSDQPLDVLRVFNDGDYQSIDLNDWIMSNPNTVLDDVFQLSPQLLDKLPKESEILIPRS

SEQ ID NO: 27 - protein, 389 aa, Synechococcus elongatus
MQKKSKFFLGLLGVITCFVLIGSFCLPSLAQTQTWRSLSNVVWGKDLPAFSYPFSKTPLVDYDGGVTKQVGTYNFPVSKGMAGVYMTLKPGAIRELHWHANAAEWAYVIEGRTRVTLTNPDGQVQIADVDQGGLWYFPRGWGHSIEGIGPGTAKFLLVFNDGTFSEGATFSITDWLSHTPISWVQQNFGWSQDEVEKLPKKQVYISRYNPEVKPLDKTQSRNPKVSRIVLPYTHNLLAEKPRTSQAGNTLKLASAKEFPASFNMAGALLRLEPGAMRQLHWHPNADEWQYVLNGSMDLAVFASEGKASMSRLQKGDVGYVPKGYGHALRNSSDQPLDVLSVFNDGDYQSIDLNDWIMSNPNTVLDDVFQLSPQLLDKLPKESEILIPRS

SEQ ID NO: 28 - protein, 389 aa, Synechococcus elongatus
MQKKSKFFLGLLGVITCFVLIGSFCLPSLAQTQTWRSLSNVVWGKDLPAFSYPFSKTPLVDYDGGVTKQVGTYNFPVSKGMAGVYMTLKPGAIRELHWHANAAEWAYVIEGRTRVTLTNPDGQVQIADVDQGGLWYFPRGWGHSIEGIGPGTAKFLLVFNDGTFSEGATFSITDWLSHTPISWVQQNFGWSQDEVEKLPKKQVYISRYNPEVKPLDKTQSRNPKVSRIVLPYTHNLLAEKPRTSQAGNTLKLASAKEFPASFNMAGALLRLEPGAMRQLHWHPNADEWQYVLNGSMDLAVFASEGKASMSRLQKGDVGYVPKGYGHALRNSSDQPLDVLTVFNDGDYQSIDLNDWIMSNPNTVLDDVFQLSPQLLDKLPKESEILIPRS

SEQ ID NO: 29 - protein, 389 aa, Synechococcus elongatus
MQKKSKFFLGLLGVITCFVLIGSFCLPSLAQTQTWRSLSNVVWGKDLPAFSYPFSKTPLVDYDGGVTKQVGTYNFPVSKGMAGVYMTLKPGAIRELHWHANAAEWAYVIEGRTRVTLTNPDGQVQIADVDQGGLWYFPRGWGHSIEGIGPGTAKFLLVFNDGTFSEGATFSITDWLSHTPISWVQQNFGWSQDEVEKLPKKQVYISRYNPEVKPLDKTQSRNPKVSRIVLPYTHNLLAEKPRTSQAGNTLKLASAKEFPASFNMAGALLRLEPGAMRQLHWHPNADEWQYVLNGSMDLAVFASEGKASMSRLQKGDVGYVPKGYGHALRNSSDQPLDVLVVFNDGDYQSIDLNDWIMSNPNTVLDDVFQLSPQLLDKLPKESEILIPRS

SEQ ID NO: 30 - protein, 389 aa, Synechococcus elongatus
MQKKSKFFLGLLGVITCFVLIGSFCLPSLAQTQTWRSLSNVVWGKDLPAFSYPFSKTPLVDYDGGVTKQVGTYNFPVSKGMAGVYMTLKPGAIRELHWHANAAEWAYVIEGRTRVTLTNPDGQVQIADVDQGGLWYFPRGWGHSIEGIGPGTAKFLLVFNDGTFSEGATFSITDWLSHTPISWVQQNFGWSQDEVEKLPKKQVYISRYNPEVKPLDKTQSRNPKVSRIVLPYTHNLLAEKPRTSQAGNTLKLASAKEFPASFNMAGALLRLEPGAMRQLHWHPNADEWQYVLNGSMDLAVFASEGKASMSRLQKGDVGYVPKGYGHALRNSSDQPLDVLWVFNDGDYQSIDLNDWIMSNPNTVLDDVFQLSPQLLDKLPKESEILIPRS

SEQ ID NO: 31 - protein, 389 aa, Synechococcus elongatus
MQKKSKFFLGLLGVITCFVLIGSFCLPSLAQTQTWRSLSNVVWGKDLPAFSYPFSKTPLVDYDGGVTKQVGTYNFPVSKGMAGVYMTLKPGAIRELHWHANAAEWAYVIEGRTRVTLTNPDGQVQIADVDQGGLWYFPRGWGHSIEGIGPGTAKFLLVFNDGTFSEGATFSITDWLSHTPISWVQQNFGWSQDEVEKLPKKQVYISRYNPEVKPLDKTQSRNPKVSRIVLPYTHNLLAEKPRTSQAGNTLKLASAKEFPASFNMAGALLRLEPGAMRQLHWHPNADEWQYVLNGSMDLAVFASEGKASMSRLQKGDVGYVPKGYGHALRNSSDQPLDVLYVFNDGDYQSIDLNDWIMSNPNTVLDDVFQLSPQLLDKLPKESEILIPRS

SEQ ID NO: 32 - protein, 389 aa, Synechococcus elongatus
MQKKSKFFLGLLGVITCFVLIGSFCLPSLAQTQTWRSLSNVVWGKDLPAFSYPFSKTPLVDYDGGVTKQVGTYNFPVSKGMAGVYMTLKPGAIRELHWHANAAEWAYVIEGRTRVTLTNPDGQVQIADVDQGGLWYFPRGWGHSIEGIGPGTAKFLLVFNDGTFSEGATFSITDWLSHTPISWVQQNFGWSQDEVEKLPKKQVYISRYNPEVKPLDKTQSRNPKVSRIVLPYTHNLLAEKPRTSQAGNTLKLASAKEFPASFNMAGALLRLEPGAMRQLHWHPNADEWQYYLNGSMDLAVFASEGKASMSRLQKGDVGYVPKGYGHALRNSSDQPLDVLIVFNDGDYQSIDLNDWIMSNPNTVLDDVFQLSPQLLDKLPKESEILIPRS

SEQ ID NO: 33 - protein, 389 aa, Synechococcus elongatus
MQKKSKFFLGLLGVITCFVLIGSFCLPSLAQTQTWRSLSNVVWGKDLPAFSYPFSKTPLVDYDGGVTKQVGTYNFPVSKGMAGVYMTLKPGAIRELHWHANAAEWAYVIEGRTRVTLTNPDGQVQIADVDQGGLWYFPRGWGHSIEGIGPGTAKFLLVFNDGTFSEGATFSITDWLSHTPISWVQQNFGWSQDEVEKLPKKQVYISRYNPEVKPLDKTQSRNPKVSRIVLPYTHNLLAEKPRTSQAGNTLKLASAKEFPASFNMAGALLRLEPGAMRQLHWHPNADEWQYVLNGSMDLAVFASEGKASMSRYQKGDVGYVPKGYGHALRNSSDQPLDVLIVFNDGDYQSIDLNDWIMSNPNTVLDDVFQLSPQLLDKLPKESEILIPRS

SEQ ID NO: 34 - protein, 389 aa, Synechococcus elongatus
MQKKSKFFLGLLGVITCFVLIGSFCLPSLAQTQTWRSLSNVVWGKDLPAFSYPFSKTPLVDYDGGVTKQVGTYNFPVSKGMAGVYMTLKPGAIRELHWHANAAEWAYVIEGRTRVTLTNPDGQVQIADVDQGGLWYFPRGWGHSIEGIGPGTAKFLLVFNDGTFSEGATFSITDWLSHTPISWVQQNFGWSQDEVEKLPKKQVYISRYNPEVKPLDKTQSRNPKVSRIVLPYTHNLLAEKPRTSQAGNTLKLASAKEFPASFNMAGALLRLEPGAMRQLHWHPNADEWQYVLNGSMDLAVFASEGKASMSRLQKGDVGYVPKGYGHALRNSSDQPLDFLIVFNDGDYQSIDLNDWIMSNPNTVLDDVFQLSPQLLDKLPKESEILIPRS

SEQ ID NO: 35 - protein, 389 aa, Synechococcus elongatus
MQKKSKFFLGLLGVITCFVLIGSFCLPSLAQTQTWRSLSNVVWGKDLPAFSYPFSKTPLVDYDGGVTKQVGTYNFPVSKGMAGVYMTLKPGAIRELHWHANAAEWAYVIEGRTRVTLTNPDGQVQIADVDQGGLWYFPRGWGHSIEGIGPGTAKFLLVFNDGTFSEGATFSITDWLSHTPISWVQQNFGWSQDEVEKLPKKQVYISRYNPEVKPLDKTQSRNPKVSRIVLPYTHNLLAEKPRTSQAGNTLKLASAKEFPASFNMAGALLRLEPGAMRQLHWHPNADEWQYYLNGSMDLAVFASEGKASMSRYQKGDVGYVPKGYGHALRNSSDQPLDVLIVFNDGDYQSIDLNDWIMSNPNTVLDDVFQLSPQLLDKLPKESEILIPRS

SEQ ID NO: 36 - protein, 389 aa, Synechococcus elongatus
MQKKSKFFLGLLGVITCFVLIGSFCLPSLAQTQTWRSLSNVVWGKDLPAFSYPFSKTPLVDYDGGVTKQVGTYNFPVSKGMAGVYMTLKPGAIRELHWHANAAEWAYVIEGRTRVTLTNPDGQVQIADVDQGGLWYFPRGWGHSIEGIGPGTAKFLLVFNDGTFSEGATFSITDWLSHTPISWVQQNFGWSQDEVEKLPKKQVYISRYNPEVKPLDKTQSRNPKVSRIVLPYTHNLLAEKPRTSQAGNTLKLASAKEFPASFNMAGALLRLEPGAMRQLHWHPNADEWQYYLNGSMDLAVFASEGKASMSRLQKGDVGYVPKGYGHALRNSSDQPLDFLIVFNDGDYQSIDLNDWIMSNPNTVLDDVFQLSPQLLDKLPKESEILIPRS

SEQ ID NO: 37 - protein, 389 aa, Synechococcus elongatus
MQKKSKFFLGLLGVITCFVLIGSFCLPSLAQTQTWRSLSNVVWGKDLPAFSYPFSKTPLVDYDGGVTKQVGTYNFPVSKGMAGVYMTLKPGAIRELHWHANAAEWAYVIEGRTRVTLTNPDGQVQIADVDQGGLWYFPRGWGHSIEGIGPGTAKFLLVFNDGTFSEGATFSITDWLSHTPISWVQQNFGWSQDEVEKLPKKQVYISRYNPEVKPLDKTQSRNPKVSRIVLPYTHNLLAEKPRTSQAGNTLKLASAKEFPASFNMAGALLRLEPGAMRQLHWHPNADEWQYVLNGSMDLAVFASEGKASMSRYQKGDVGYVPKGYGHALRNSSDQPLDFLIVFNDGDYQSIDLNDWIMSNPNTVLDDVFQLSPQLLDKLPKESEILIPRS

SEQ ID NO: 38 - protein, 389 aa, Synechococcus elongatus
MQKKSKFFLGLLGVITCFVLIGSFCLPSLAQTQTWRSLSNVVWGKDLPAFSYPFSKTPLVDYDGGVTKQVGTYNFPVSKGMAGVYMTLKPGAIRELHWHANAAEWAYVIEGRTRVTLTNPDGQVQIADVDQGGLWYFPRGWGHSIEGIGPGTAKFLLVFNDGTFSEGATFSITDWLSHTPISWVQQNFGWSQDEVEKLPKKQVYISRYNPEVKPLDKTQSRNPKVSRIVLPYTHNLLAEKPRTSQAGNTLKLASAKEFPASFNMAGALLRLEPGAMRQLHWHPNADEWQYYLNGSMDLAVFASEGKASMSRYQKGDVGYVPKGYGHALRNSSDQPLDFLIVFNDGDYQSIDLNDWIMSNPNTVLDDVFQLSPQLLDKLPKESEILIPRS

SEQ ID NO: 39 - protein, 389 aa, Synechococcus elongatus
MQKKSKFFLGLLGVITCFVLIGSFCLPSLAQTQTWRSLSNVVWGKDLPAFSYPFSKTPLVDYDGGVTKQVGTYNFPVSKGMAGVYMTLKPGAIRELHWHANAAEWAYVIEGRTRVTLTNPDGQVQIADVDQGGLWYFPRGWGHSIEGIGPGTAKFLLVFNDGTFSEGATFSITDWLSHTPISWVQQNFGWSQDKVEKLPKKQVYISRYNPEVKPLDKTQSRNPKVSRIVLPYTHNLLAEKPRTSQAGNTLKLASAKEFPASFNMAGALLRLEPGAMRQLHWHPNADEWQYYLNGSMDLAVFASEGKASMSRYQKGDVGYVPKGYGHALRNSSDQPLDFLIVFNDGDYQSIDLNDWIMSNPNTVLDDVFQLSPQLLDKLPKESEILIPRS

SEQ ID NO: 40 - protein, 394 aa, Synechococcus elongatus
MVNSVIGWLRRRFLLVGLSVLLITFLGIFTPTIAQSEQWRSLSNVVWGKDLPAFTYAFSKTPLVLYDGGTTKQVGTYNFPVSKGMAGVYMSLEPGAIRELHWHANAAEWAYVMEGRTRITLTSPEGKVEIADVDKGGLWYFPRGWGHSIEGIGPDTAKFLLVFNDGTFSEGATFSVTDWLSHTPIAWVEENLGWTAAQVAQLPKKQVYISSYGPASGPLASATPQGQTAKIEVPHTHNLLGQQPLVSLGGNELRLASAKEFPGSFNMTGALIHLEPGAMRQLHWHPNADEWQYVLDGEMDLTVFASEGKASVSRLQQGDVGYVPKGYGHAIRNSSQKPLDIVVVFNDGDYQSIDLSTWLASNPSSVLGNTFQISPELTKKLPVQDTIFSLPTQP

SEQ ID NO: 41 - protein, 394 aa, Bacillus clausii
MKRGDNVKPLKGNPNIPQPIRADGAGGVDRGPRNLMRDLQNPNILVPPETDRGLIPNLRFSFSDAHMQLNHGGWSREITQRDLPIATTLAGVNMSLTPGGVRELHWHKQAEWSYMLLGHARITAVDQNGRNFIADVGPGDLWYFPPGIPHSIQGLDDGCEFLLVFDDGMFSDLSTLSLSDWMAHTPKDVLSANFGVPESVFATIPTEQVYIYQDEVPGPLQSQQINSPYGAVPQTFKHELLKQPPLVTPGGSVRIVDSRNFPVSKTIAAALVEVEPGAMREMHWHPNNDEWQYYLTGQARMTVFTGNGVARTFDYRAGDVGYVPFATGHYIQNTGNESVWFLEMFKSDRFEDVSLNQWLALTPTELVQHNIHVDSKFTNKLRKEKWPVVKYPTI

SEQ ID NO: 42 - protein, 470 aa, Agrocybe aegerita
MISVASCTIALLLSSVAFAAPAPSSAASSIVVSATSSSTVSSAPVSVSSFLPTTSIAAATPSSIAVALSSTATVPFIDLNPNGPLWDPSVSGVPQAERGSLGATIMGPTDVDTTKANPDLLAPPTTDHGSVDNAKWAFSLSHNRLQTGGWAREQNIGAMPIATEMASVNMRLEPGAIRELHWHKTAEWAYVLKGNTQVTAVDQNGKNFIGTVGPGDLWYFPPGIPHSLQATGDDPEGSEFILVFDSGAFSEDSTFLLTDWMSHVPVEVLAKNFQTDISAFARIPAEELYIFPAAVPPDSQQDPTSPEGTVPNPFTFALSKVPPMQLSGGTAKIVDSTTFTVSKAIAAAEVTIEPGAIRELHWHPTQDEWSFFIEGRARMTIFAAQSNARTFDYQAGDIGYVPATMGHYVENIGNTTVRYLEIFNTAVFEDISLSNWLALTPPELVKAHLGFDDATMAHLAKVKPIVVGPA

SEQ ID NO: 43 - protein, 452 aa, Agrocybe aegerita
MAPAPSSAASSIVVSATSSSTVSSAPVSVSSFLPTTSIAAATPSSIAVALSSTATVPFIDLNPNGPLWDPSVSGVPQAERGSLGATIMGPTDVDTTKANPDLLAPPTTDHGSVDNAKWAFSLSHNRLQTGGWAREQNIGAMPIATEMASVNMRLEPGAIRELHWHKTAEWAYVLKGNTQVTAVDQNGKNFIGTVGPGDLWYFPPGIPHSLQATGDDPEGSEFILVFDSGAFSEDSTFLLTDWMSHVPVEVLAKNFQTDISAFARIPAEELYIFPAAVPPDSQQDPTSPEGTVPNPFTFALSKVPPMQLSGGTAKIVDSTTFTVSKAIAAAEVTIEPGAIRELHWHPTQDEWSFFIEGRARMTIFAAQSNARTFDYQAGDIGYVPATMGHYVENIGNTTVRYLEIFNTAVFEDISLSNWLALTPPELVKAHLGFDDATMAHLAKVKPIVVGPA

SEQ ID NO: 44 - protein, 386 aa, Bacillus amyloliquefaciens
MSKENNCNIPQPIRGDKGATVTIPRNLERDRQNPDMLTPPETDHGTVDNMKFSFSDVHNRLEKGGYAREVTVRELPISENLASVNMRLKPGAIRELHWHKEAEWAYMLTGKARVTIVDEQGRSFIDDVKEGDLWYFPSGLPHSIQALKEGCEFLLVFDDGSFSENSTFQVTDWLAHTPLDVIASNFGVSEKDLAGLPGKEKYIFEEPVPGKLKDDIVEGPNGEVPYPFTYRLLDEGPTAETDGGKVYIADSTNFKVSKTIASALVVVEPGAMRELHWHPNTHEWQYYISGKGRMTVFASDGHARTFNYQAGDVGYVPFAMGHYVENLGDEPLVFLEIFKDDHYADVSLNQWLAMLPEKFVQQHLDLGKDFTDILSKEKHPVVKKKC

SEQ ID NO: 45 - protein, 387 aa, Bacillus pumilus
MSEKQNGVPQPIRGEKGATVKIPRNLERDRQNPDMLTPPETDHGTVPNMKYSFSDTHNRLEKGGYAREVTVRELPISKSLASVNMRLKPGAIRELHWHKEAEWAYMIYGEARITSVDAEGRNFTEDVTEGDLWYFPSGLPHSIQALEPGAEFLLVFDDGSFSENSTFQVTDWLAHTPEEVVLQNFGMTKEQFEKLPEKEKYIFQKGIPGSLECDKVKTGQGEVPNSFKYELLKQEPITSSGGQVWIADSTNFKASKTIASALVKVDPGAIRELHWHPNTDEWQYFISGKARMTVFASDGHARTFNYQAGDVGYVPFAMGHYVENTGDEPLYFLEIFKSDHYADISLNQWLAVTPKQLILDHLDQGEEFLKLLDTEKHPVIAAPKKED

SEQ ID NO: 46 - protein, 402 aa, Clostridium botulinum
MYIQNQYQNLCNLLMSGCIPQPIRDGAGATDIGPRDILRDLENPDMLVPPSTDTGLIPNLKFSFSDTNMTIRPGGWSREITVRELPIATTMAGVNMRLTPGGVREVHWHQQSEWSYMLKGSARITAVDDRGRNFIADIGPGDLWFFPPLFPHSIQGLEEGCEFLLLFDDGNFSDLRTFSLSEFFAHYPKDVLAANFGVTKNCFNCLPEGQVYIYQDTIPGPLESEAIESPYGTIPQSYKHSLLAQKPMTTPGGSVRIADTSNFPVAKTTAAALVEIKPGGMREIHWHPNDEFQYFLTGQSRMTVFADTGASRTFDYRAGDVGYVPTGYGHYVQNIGNETVWFLEAFRSDRFKSISLSQMMAITPQQLIASNLNVGPGFLNALSRSKFQCSVGPCFHQTECSD

SEQ ID NO: 47 - protein, 385 aa, Bacillus subtilis
MKKQNDIPQPIRGDKGATVKIPRNIERDRQNPDMLVPPETDHGTVSNMKFSFSDTHNRLEKGGYAREVTVRELPISENLASVNMRLKPGAIRELHWHKEAEWAYMIYGSARVTIVDEKGRSFIDDVGEGDLWYFPSGLPHSIQALEEGAEFLLVFDDGSFSENSTFQLTDWLAHTPKEVIAANFGVTKEEISNLPGKEKYIFENQLPGSLKDDIVEGPNGEVPYPFTYRLLEQEPIESEGGKVYIADSTNFKVSKTIASALVTVEPGAMRELHWHPNTHEWQYYISGKARMTVFASDGHARTFNYQAGDVGYVPFAMGHYVENIGDEPLVFLEIFKDDHYADVSLNQWLAMLPETFVQAHLDLGKDFTDVLSKEKHPVVKKKCSK

SEQ ID NO: 48 - protein, 401 aa, Synechococcus elongatus
MASLSRLFKPYSQLFSKFRLFLICLVLLLIGSSCWLLPALSQSSQWHSLSGVVWGKDLPAFSYPFHQTPLTLYDGGTTKQVGTYNFPVSKGMAGVYMTLEPGAIRELHWHANAAEWAYVISGRTRITLTSPDGNVQIADVDQGGLWYFPRGWGHSIEGLGPGTAKFILVFNDGTFSEGATFSITDWVSHMPISWVQDALGLTATQVQGLPNKQVYISRRPPAPGPLATTQPRNPNIPRLEVTHVHDLAAQPFFAVEDQNTILLASNKEFPASFNMAGGIIHLEPGAIRQPHWHPNADEWQYILDGEMELTVFASEGKASISTLKTGDVGYIPKGYGHALRNPSHKPMDVLLVFDAGEYESIELTGWIASNPDSVVGNTFQVPANLLSRLPRQKKLFARPGK

SEQ ID NO: 49 - protein, 410 aa, Agrocybe aegerita
  MOD_RES (401)..(401): Any amino acid
PSSIAVALSSTATVPFIDLNPNGPLWDPSVSGVPQAERGSLGATIMGPTDVDTTKANPDLLAPPTTDHGSVDNAKWAFSLSHNRLQTGGWAREQNIGAMPIATEMASVNMRLEPGAIRELHWHKTAEWAYVLKGNTQVTAVDQNGKNFIGTVGPGDLWYFPPGIPHSLQATGDDPEGSEFILVFDSGAFSEDSTFLLTDWMSHVPVEVLAKNFQTDISAFARIPAEELYIFPAAVPPDSQQDPTSPEGTVPNPFTFALSKVPPMQLSGGTAKIVDSTTFTVSKAIAAAEVTIEPGAIRELHWHPTQDEWSFFIEGRARMTIFAAQSNARTFDYQAGDIGYVPATMGHYVENIGNTTVRYLEIFNTAVFEDISLSNWLALTPPELVKAHLGFDDATMAHLAXVKPIVVGPA

SEQ ID NO: 50 - protein, 391 aa, Bacillus cereus
MKKRTVNEAGRNVPQPIRSDGAGAIDSGPRNVMRDIQNPNMLVPPITDAGLVPNLKFSFSDTSMILKQGGWSREITVRELPVSTTIAGVNMSLTAGGVRELHWHKEAEWAYMLLGRARITAVDQNGRNFIADVGPGDLWYFPPGIPHSIQGLEHCEFLLVFDDGHFSDLSTLAISDWFAHTPKEVLSANFGVPESAFRSIPSDQVYIYQGEVPGSLESQEVQSPKGEVPLTFKHELLKQKPIKTPGGSVRIVDSTNFPISKTIAAALVEVEPGGMRELHWHPNNDEWQYYLTGEARMTVFLGNGTARTFDYRAGDVGYVPFATGHYIQNTGTETLWFLEMFRSNRFEDVSLNQWMALTPKEIVESNIHVGPQVMDALRKEKWPVVKYPGFS

SEQ ID NO: 51 - protein, 386 aa, Bacillus pumilus
MSEKQNGVPQPIRGEKGATVKIPRNLERDRQNPDMLTPPETDHGTVPNMKYSFSDTHNRLEKGGYAREVTVRELPISKSLASVNMRLKPGAIRELHWHKEAEWAYMIYGEARITSVDAEGRNFTEDVTEGDLWYFPSGLPHSIQALEPGAEFLLVFDDGSFSENSTFQVTDWLAHTPEEVVLQNFGMTKEQFEKLPEKEKYIFQKGIPGSLECDKVKTEQGEVPNSFKYELLKQEPITSSGGQVWIADSTNFKASKTIASALVKVDPGAIRELHWHPNTDEWQYFISGKARMTVFASDGHARTFNYQAGDVGYVPFAMGHYVENTGDEPLYFLEIFKSDHYADISLNQWLAVTPKQLVLDHLDQGEDFLKLLDTEKHPVIAAPKKE

SEQ ID NO: 52 - protein, 386 aa, Bacillus amyloliquefaciens
MSKENNCNIPQPIRGDKGATVTIPRNLERDRQNPDMLTPPETDHGTVDNMKFSFSDVHNRLEKGGYAREVTVRELPISENLASVNMRLKPGAIRELHWHKEAEWAYMLTGKARVTIVDEQGRSFIDDVKEGDLWYFPSGLPHSIQALKEGCEFLLVFDDGSFSENSTFQVTDWLAHTPLDVIANNFGVSEKDLAGLPGKEKYIFEEPVPGKLKDDIVEGPNGEVPYPFTYRLLDEGPTAETDGGKVYIADSTNFKVSKTIASALVVVEPGAMRELHWHPNTHEWQYYISGKGRMTVFASDGHARTFNYQAGDVGYVPFAMGHYVENLGDEPLVFLEIFKDDHYADVSLNQWLAMLPEKFVQQHLDLGKDFTDILSKEKHPVVKKKC

SEQ ID NO: 53 - protein, 8 aa, Synechococcus elongatus
  MOD_RES (4)..(7): Any amino acid
HWHXXXXE